European Patent Specification EP 3 701 048 B1, published August 6, 2025. Title: METHODS AND COMPOSITIONS FOR ASSESSING AND TREATING INTRAOCULAR DISEASES AND DISORDERS. Applicant: Zhuhai Qiwei Bio-technology Ltd. The sequence listing filed with the application follows.

SEQUENCE LISTING (52 sequences)

SEQ ID NO: 1 - DNA, 23 bp, Artificial Sequence
gattggtttactacccgtgagcg

SEQ ID NO: 2 - DNA, 21 bp, Artificial Sequence
atagcagggattccagcgaca

SEQ ID NO: 3 - DNA, 17 bp, Artificial Sequence
ggttcaatgagcctact

SEQ ID NO: 4 - DNA, 14 bp, Artificial Sequence
gccagcgtctttcc

SEQ ID NO: 5 - DNA, 19 bp, Artificial Sequence
tcccgtcttcatctactgc

SEQ ID NO: 6 - DNA, 17 bp, Artificial Sequence
ggacgcctactggacaa

SEQ ID NO: 7 - DNA, 17 bp, Artificial Sequence
ccgcacaggttgtccca

SEQ ID NO: 8 - DNA, 18 bp, Artificial Sequence
ctgctgcgttgtcgttcc

SEQ ID NO: 9 - DNA, 18 bp, Artificial Sequence
tggtgcgatggcgatgtt

SEQ ID NO: 10 - DNA, 18 bp, Artificial Sequence
ggttgcggcatgtgcttt

SEQ ID NO: 11 - DNA, 17 bp, Artificial Sequence
gcgttcgtccgctgtca

SEQ ID NO: 12 - DNA, 19 bp, Artificial Sequence
ggcaacccgctagaatccc

SEQ ID NO: 13 - DNA, 19 bp, Artificial Sequence
tagtggataatgccgttga

SEQ ID NO: 14 - DNA, 15 bp, Artificial Sequence
cggtttgccagaagc

SEQ ID NO: 15 - DNA, 18 bp, Artificial Sequence
gttacactgctccgacaa

SEQ ID NO: 16 - DNA, 16 bp, Artificial Sequence
ttcgcatcagcaataa

SEQ ID NO: 17 - DNA, 14 bp, Artificial Sequence
gctggctcctttgg

SEQ ID NO: 18 - DNA, 16 bp, Artificial Sequence
gcattactgcctggtg

SEQ ID NO: 19 - DNA, 15 bp, Artificial Sequence
gactccgacttgttt

SEQ ID NO: 20 - DNA, 19 bp, Artificial Sequence
cattatctggcgttttagc

SEQ ID NO: 21 - DNA, 17 bp, Artificial Sequence
gaagcggagttcaaagg

SEQ ID NO: 22 - DNA, 18 bp, Artificial Sequence
atggcaaatcaccaatca

SEQ ID NO: 23 - DNA, 21 bp, Artificial Sequence
gaccaggtagccgtcgttctc

SEQ ID NO: 24 - DNA, 21 bp, Artificial Sequence
tgctgaccctgaccgacattc

SEQ ID NO: 25 - DNA, 20 bp, Artificial Sequence
gaagtgcgtgcgtatagtgt

SEQ ID NO: 26 - DNA, 19 bp, Artificial Sequence
aaagaacgaccaagtgctg

SEQ ID NO: 27 - DNA, 18 bp, Artificial Sequence
ttgaagtgaaacgtcctc

SEQ ID NO: 28 - DNA, 17 bp, Artificial Sequence
tgtctcatctaaccacc

SEQ ID NO: 29 - DNA, 16 bp, Artificial Sequence
tggagcgattataccg

SEQ ID NO: 30 - DNA, 16 bp, Artificial Sequence
gtacccgcttgattga

SEQ ID NO: 31 - DNA, 20 bp, Artificial Sequence
agcgggaaatcgtgcgtgac

SEQ ID NO: 32 - DNA, 21 bp, Artificial Sequence
caggcagctcgtagctcttct

SEQ ID NO: 33 - DNA, 17 bp, Artificial Sequence
cctgcccttgactttgg

SEQ ID NO: 34 - DNA, 16 bp, Artificial Sequence
aagccgcgagtccatc

SEQ ID NO: 35 - DNA, 18 bp, Artificial Sequence
cgggaaatcgtgcgtgac

SEQ ID NO: 36 - DNA, 17 bp, Artificial Sequence
atcgggcagctcgtagc

SEQ ID NO: 37 - DNA, 18 bp, Artificial Sequence
cttactacagcggcaacg

SEQ ID NO: 38 - DNA, 17 bp, Artificial Sequence
ccatccagagggcagag

SEQ ID NO: 39 - DNA, 17 bp, Artificial Sequence
caaggctgatgggaacg

SEQ ID NO: 40 - DNA, 22 bp, Artificial Sequence
cacggacaccagtatcttctcc

SEQ ID NO: 41 - DNA, 17 bp, Artificial Sequence
gctgctcctggtgttgc

SEQ ID NO: 42 - DNA, 17 bp, Artificial Sequence
tgccgtcgaggatgtac

SEQ ID NO: 43 - DNA, 17 bp, Artificial Sequence
ctccagtggctgaaccg

SEQ ID NO: 44 - DNA, 20 bp, Artificial Sequence
tgaagaggacctgggagtag

SEQ ID NO: 45 - DNA, 17 bp, Artificial Sequence
gaatgtccaacgcaaag

SEQ ID NO: 46 - DNA, 19 bp, Artificial Sequence
ctcgaaacatctgactcct

SEQ ID NO: 47 - DNA, 15 bp, Artificial Sequence
cgagatgcgtcaaag

SEQ ID NO: 48 - DNA, 18 bp, Artificial Sequence
cttactggtaacagggtc

SEQ ID NO: 49 - DNA, 18 bp, Artificial Sequence
gcgtagaccatactttcc

SEQ ID NO: 50 - DNA, 16 bp, Artificial Sequence
gtgaccacccatcttg

SEQ ID NO: 51 - DNA, 40 bp, Artificial Sequence
gcatgatgatttgacgtcatccccaccttcctccggtttg

SEQ ID NO: 52 - DNA, 20 bp, Artificial Sequence
tacgtccttacggttactcc